European Patent Application EP 4 760 726 A1, published June 17, 2026. Title: 一种用于鉴定与MHC-I/HLA-I类结合及TCR识别肽段的方法、设备及存储介质. Applicant: 北京立康生命科技有限公司. Application CN. The sequence listing filed with the application follows.

SEQUENCE LISTING (6 sequences)

SEQ ID NO: 1 - protein, 23 aa, synthetic construct
MAFSAEDVLKEYDRRRRMEALLL

SEQ ID NO: 2 - protein, 40 aa, synthetic construct
MIINPTSDPEVSALEKKNTGRIAQIIGPVLDVTFPPGKMP

SEQ ID NO: 3 - protein, 8 aa, synthetic construct
EIEICDGF

SEQ ID NO: 4 - protein, 105 aa, synthetic construct
MRVTAPRTLLLLLWGAVALTETWAGSHSMRYFHTSVSRPGRGEPRFITVGYVDDTAGLAVLAVVVIGAVVAAVMCRRKSSGGKGGSYSQAACSDSAQGSDVSLTA

SEQ ID NO: 5 - protein, 9 aa, synthetic construct
KAISKNVLF

SEQ ID NO: 6 - protein, 10 aa, synthetic construct
RPTRPDKARR